European Patent Specification EP 3 800 199 B1, published August 21, 2024. Title: H3.3 CTL PEPTIDES AND USES THEREOF. Applicant: The Regents of the University of California. The sequence listing filed with the application follows.

SEQUENCE LISTING (17 sequences)

SEQ ID NO: 1 - protein, 10 aa, Artificial Sequence
  synthetic peptide construct
  MOD_RES (1)..(1): Xaa is Arg or Ala
  MOD_RES (1)..(1): Xaa is Arg or Ala; when Xaa is Arg, citrullination of Arg may be present or absent
  MOD_RES (6)..(6): Xaa is Ser or Ala
XMSAPXTGGV

SEQ ID NO: 2 - protein, 10 aa, Artificial Sequence
  synthetic peptide construct
RMSAPSTGGV

SEQ ID NO: 3 - protein, 10 aa, Artificial Sequence
  synthetic peptide construct
RKSAPSTGGV

SEQ ID NO: 4 - protein, 10 aa, Artificial Sequence
  synthetic peptide construct
RMSAPSTGGV

SEQ ID NO: 5 - protein, 10 aa, Artificial Sequence
  synthetic peptide construct
AMSAPSTGGV

SEQ ID NO: 6 - protein, 10 aa, Artificial Sequence
  synthetic peptide construct
RMSAPATGGV

SEQ ID NO: 7 - protein, 10 aa, Artificial Sequence
  synthetic peptide construct
AMSAPATGGV

SEQ ID NO: 8 - protein, 273 aa, Artificial Sequence
  synthetic peptide construct
MLTASLLRAVIASICVVSSMAQKVTQAQTEISVVEKEDVTLDCVYETRDTTYYLFWYKQPPSGELVFLIRRNSFDEQNEISGRYSWNFQKSTSSFNFTITASQVVDSAVYFCALSEENDMRFGAGTRLTVKPNIQNPDPAVYQLRDSKSSDKSVCLFTDFDSQTNVSQSKDSDVYITDKTVLDMRSMDFKSNSAVAWSNKSDFACANAFNNSIIPEDTFFPSPESSCDVKLVEKSFETDTNLNFQNLSVIGFRILLLKVAGFNLLMTLRLWSS

SEQ ID NO: 9 - DNA, 822 bp, Artificial Sequence
  synthetic nucleotide sequence
atgctgactgccagcctgttgagggcagtcatagcctccatctgtgttgtatccagcatggctcagaaggtaactcaagcgcagactgaaatttctgtggtggagaaggaggatgtgaccttggactgtgtgtatgaaacccgtgatactacttattacttattctggtacaagcaaccaccaagtggagaattggttttccttattcgtcggaactcttttgatgagcaaaatgaaataagtggtcggtattcttggaacttccagaaatccaccagttccttcaacttcaccatcacagcctcacaagtcgtggactcagcagtatacttctgtgctctgagtgaggagaatgacatgcgctttggagcagggaccagactgacagtaaaaccaaatatccagaaccctgaccctgccgtgtaccagctgagagactctaaatccagtgacaagtctgtctgcctattcaccgattttgattctcaaacaaatgtgtcacaaagtaaggattctgatgtgtatatcacagacaaaactgtgctagacatgaggtctatggacttcaagagcaacagtgctgtggcctggagcaacaaatctgactttgcatgtgcaaacgccttcaacaacagcattattccagaagacaccttcttccccagcccagaaagttcctgtgatgtcaagctggtcgagaaaagctttgaaacagatacgaacctaaactttcaaaacctgtcagtgattgggttccgaatcctcctcctgaaagtggccgggtttaatctgctcatgacgctgcggctgtggtccagctga

SEQ ID NO: 10 - protein, 311 aa, Artificial Sequence
  synthetic peptide construct
MGPQLLGYVVLCLLGAGPLEAQVTQNPRYLITVTGKKLTVTCSQNMNHEYMSWYRQDPGLGLRQIYYSMNVEVTDKGDVPEGYKVSRKEKRNFPLILESPNPNQTSLYFCASGWGGPFYEQYFGPGTRLTVTEDLKNVFPPEVAVFEPSEAEISHTQKATLVCLATGFYPDHVELSWWVNGKEVHSGVSTDPQPLKEQPALNDSRYCLSSRLRVSATFWQNPRNHFRCQVQFYGLSENDEWTQDRAKPVTQIVSAEAWGRADCGFTSESYQQGVLSATILYEILLGKATLYAVLVSALVLMAMVKRKDSRG

SEQ ID NO: 11 - DNA, 936 bp, Artificial Sequence
  synthetic nucleotide sequence
atgggcccccagctccttggctatgtggtcctttgccttctaggagcaggccccctggaagcccaagtgacccagaacccaagatacctcatcacagtgactggaaagaagttaacagtgacttgttctcagaatatgaaccatgagtatatgtcctggtatcgacaagacccagggctgggcttaaggcagatctactattcaatgaatgttgaggtgactgataagggagatgttcctgaagggtacaaagtctctcgaaaagagaagaggaatttccccctgatcctggagtcgcccaaccccaaccagacctctctgtacttctgtgccagcggctggggtggtccattctacgagcagtacttcgggccgggcaccaggctcacggtcacagaggacctgaaaaacgtgttcccacccgaggtcgctgtgtttgagccatcagaagcagagatctcccacacccaaaaggccacactggtatgcctggccacaggcttctaccccgaccacgtggagctgagctggtgggtgaatgggaaggaggtgcacagtggggtcagcacagacccgcagcccctcaaggagcagcccgccctcaatgactccagatactgcctgagcagccgcctgagggtctcggccaccttctggcagaacccccgcaaccacttccgctgtcaagtccagttctacgggctctcggagaatgacgagtggacccaggatagggccaaacccgtcacccagatcgtcagcgccgaggcctggggtagagcagactgtggcttcacctccgagtcttaccagcaaggggtcctgtctgccaccatcctctatgagatcttgctagggaaggccaccttgtatgccgtgctggtcagtgccctcgtgctgatggccatggtcaagagaaaggattccagaggctag

SEQ ID NO: 12 - protein, 7 aa, Artificial Sequence
  synthetic peptide construct
TRDTTYY

SEQ ID NO: 13 - protein, 4 aa, Artificial Sequence
  synthetic peptide construct
RNSF

SEQ ID NO: 14 - protein, 4 aa, Artificial Sequence
  synthetic peptide construct
ALSE

SEQ ID NO: 15 - protein, 6 aa, Artificial Sequence
  synthetic peptide construct
NMNHEY

SEQ ID NO: 16 - protein, 8 aa, Artificial Sequence
  synthetic peptide construct
YSMNVEVT

SEQ ID NO: 17 - protein, 13 aa, Artificial Sequence
  synthetic peptide construct
CASGWGGPFYEQY